European Patent Application EP 4 600 358 A1, published August 13, 2025. Title: COMPOUND FOR INHIBITING C3 GENE EXPRESSION, PHARMACEUTICAL COMPOSITION, AND USE THEREOF. Applicant: RIGERNA THERAPEUTICS (SUZHOU) CO., LTD. Application CN PCT/CN2024/086555, filed April 8, 2024. The sequence listing filed with the application follows.

SEQUENCE LISTING (28 sequences)

SEQ ID NO: 1 - RNA, 19 nt, synthetic construct
  source 1..19: mol_type = other RNA
cagagaaattctactacat

SEQ ID NO: 2 - RNA, 21 nt, synthetic construct
  source 1..21: mol_type = other RNA
atgtagtagaatttctctgta

SEQ ID NO: 3 - RNA, 19 nt, synthetic construct
  source 1..19: mol_type = other RNA
aaattctactacatctata

SEQ ID NO: 4 - RNA, 21 nt, synthetic construct
  source 1..21: mol_type = other RNA
tatagatgtagtagaatttct

SEQ ID NO: 5 - RNA, 19 nt, synthetic construct
  source 1..19: mol_type = other RNA
cgaagctcatgaatatatt

SEQ ID NO: 6 - RNA, 21 nt, synthetic construct
  source 1..21: mol_type = other RNA
aatatattcatgagcttcgta

SEQ ID NO: 7 - RNA, 19 nt, synthetic construct
  source 1..19: mol_type = other RNA
caactcacctgtaataaat

SEQ ID NO: 8 - RNA, 21 nt, synthetic construct
  source 1..21: mol_type = other RNA
atttattacaggtgagttgat

SEQ ID NO: 9 - RNA, 19 nt, synthetic construct
  source 1..19: mol_type = other RNA
gagaattgcttcatacaaa

SEQ ID NO: 10 - RNA, 21 nt, synthetic construct
  source 1..21: mol_type = other RNA
tttgtatgaagcaattctcct

SEQ ID NO: 11 - DNA, 21 bp, synthetic construct
  source 1..21: mol_type = other DNA
agtctcctgctttagtgatgc

SEQ ID NO: 12 - DNA, 20 bp, synthetic construct
  source 1..20: mol_type = other DNA
gcctttgttctcatctcgct

SEQ ID NO: 13 - DNA, 27 bp, synthetic construct
  source 1..27: mol_type = other DNA
ctgttgacctgctcctcgcaaatatct

SEQ ID NO: 14 - DNA, 19 bp, synthetic construct
  source 1..19: mol_type = other DNA
aagaaggtggtgaagcagg

SEQ ID NO: 15 - DNA, 18 bp, synthetic construct
  source 1..18: mol_type = other DNA
caaagtggtcgttgaggg

SEQ ID NO: 16 - DNA, 18 bp, synthetic construct
  source 1..18: mol_type = other DNA
caacagcgacacccactc

SEQ ID NO: 17 - DNA, 20 bp, synthetic construct
  source 1..20: mol_type = other DNA
tcctgcgatcagaagagacc

SEQ ID NO: 18 - DNA, 20 bp, synthetic construct
  source 1..20: mol_type = other DNA
gacctttggccttagcatgg

SEQ ID NO: 19 - DNA, 21 bp, synthetic construct
  source 1..21: mol_type = other DNA
accgacaaggtgccttggcct

SEQ ID NO: 20 - DNA, 20 bp, synthetic construct
  source 1..20: mol_type = other DNA
tcgtggaaggactcatgacc

SEQ ID NO: 21 - DNA, 20 bp, synthetic construct
  source 1..20: mol_type = other DNA
gcagggatgatgttctggag

SEQ ID NO: 22 - DNA, 20 bp, synthetic construct
  source 1..20: mol_type = other DNA
ctccgcggccatcacgccac

SEQ ID NO: 23 - DNA, 21 bp, synthetic construct
  source 1..21: mol_type = other DNA
agtctcctgctttagtgatgc

SEQ ID NO: 24 - DNA, 20 bp, synthetic construct
  source 1..20: mol_type = other DNA
gcctttgttctcatctcgct

SEQ ID NO: 25 - DNA, 25 bp, synthetic construct
  source 1..25: mol_type = other DNA
ctgttgacctgctcctcgcaaatat

SEQ ID NO: 26 - DNA, 18 bp, synthetic construct
  source 1..18: mol_type = other DNA
ccttccgtgttcctaccc

SEQ ID NO: 27 - DNA, 18 bp, synthetic construct
  source 1..18: mol_type = other DNA
gagacaacctggtcctca

SEQ ID NO: 28 - DNA, 18 bp, synthetic construct
  source 1..18: mol_type = other DNA
ccgcctggagaaacctgc